European Patent Application EP 4 166 564 A1, published April 19, 2023. Title: Peptide Having Botulinum Toxin-Like Activity and Uses thereof. Applicant: CAREGEN CO., LTD. The sequence listing filed with the application follows.

SEQUENCE LISTING (9 sequences)

SEQ ID NO: 1 - protein, 5 aa, Artificial Sequence
  Peptide
KFLIK

SEQ ID NO: 2 - DNA, 20 bp, Artificial Sequence
  Forward primer for Col1a1
caccctcaagagcctgagtc

SEQ ID NO: 3 - DNA, 20 bp, Artificial Sequence
  Reverse primer for Col1a1
agacggctgagtagggaaca

SEQ ID NO: 4 - DNA, 20 bp, Artificial Sequence
  Forward primer for Fibronectin
ccaggaaccgagtacaccat

SEQ ID NO: 5 - DNA, 20 bp, Artificial Sequence
  Reverse primer for Fibronectin
atacccaggttgggtgatga

SEQ ID NO: 6 - DNA, 20 bp, Artificial Sequence
  Forward primer for Elastin
ggacccctgactcgcgacct

SEQ ID NO: 7 - DNA, 20 bp, Artificial Sequence
  Reverse primer for Elastin
ggggaggtgggactgcccaa

SEQ ID NO: 8 - DNA, 25 bp, Artificial Sequence
  Forward primer for GAPDH
ggtgtgaacggatttggccgtattg

SEQ ID NO: 9 - DNA, 25 bp, Artificial Sequence
  Reverse primer for GAPDH
ccgttgaatttgccgtgagtggagt